European Patent Application EP 4 206 328 A1, published July 5, 2023. Title: YEAST POWDER RICH IN NICOTINAMIDE MONONUCLEOTIDE (NMN), AND PREPARATION METHOD AND APPLICATIONS THEREOF. Applicant: TCI CO., LTD. Application EP 21860450.2, filed August 25, 2021. The sequence listing filed with the application follows.

SEQUENCE LISTING (27 sequences)

SEQ ID NO: 1 - DNA, 22 bp, synthetic construct
  misc_feature 1..22: note = PARP2-F
  source 1..22: mol_type = other DNA
agcaagatgaatctgtgaaggc

SEQ ID NO: 2 - DNA, 20 bp, synthetic construct
  misc_feature 1..20: note = PARP2-R
  source 1..20: mol_type = other DNA
cactgaagttcctctgggca

SEQ ID NO: 3 - DNA, 19 bp, synthetic construct
  misc_feature 1..19: note = CCT5-F
  source 1..19: mol_type = other DNA
ataaatgtgaggctgaatc

SEQ ID NO: 4 - DNA, 18 bp, synthetic construct
  misc_feature 1..18: note = CCT5-R
  source 1..18: mol_type = other DNA
acttgtcacttgtggcac

SEQ ID NO: 5 - DNA, 21 bp, synthetic construct
  misc_feature 1..21: note = CCT6A-F
  source 1..21: mol_type = other DNA
tgtgtatcttaatccagactc

SEQ ID NO: 6 - DNA, 20 bp, synthetic construct
  misc_feature 1..20: note = CCT6A-R
  source 1..20: mol_type = other DNA
cgtttcacctaagagttgtc

SEQ ID NO: 7 - DNA, 24 bp, synthetic construct
  misc_feature 1..24: note = CCT7-F
  source 1..24: mol_type = other DNA
gtggcatggacaagcttattgtag

SEQ ID NO: 8 - DNA, 19 bp, synthetic construct
  misc_feature 1..19: note = CCT7-R
  source 1..19: mol_type = other DNA
cagaattgtggccccatca

SEQ ID NO: 9 - DNA, 17 bp, synthetic construct
  misc_feature 1..17: note = CCT8-F
  source 1..17: mol_type = other DNA
acccggaggtggagcaa

SEQ ID NO: 10 - DNA, 25 bp, synthetic construct
  misc_feature 1..25: note = CCT8-R
  source 1..25: mol_type = other DNA
ggacatgtctctccatatgatgtga

SEQ ID NO: 11 - DNA, 20 bp, synthetic construct
  misc_feature 1..20: note = Parkin-F
  source 1..20: mol_type = other DNA
gcagagaccgtggagaaaag

SEQ ID NO: 12 - DNA, 20 bp, synthetic construct
  misc_feature 1..20: note = Parkin-R
  source 1..20: mol_type = other DNA
cttttctccacggtctctgc

SEQ ID NO: 13 - DNA, 23 bp, synthetic construct
  misc_feature 1..23: note = Atg1-F
  source 1..23: mol_type = other DNA
caggaggacgagaacacggtgtc

SEQ ID NO: 14 - DNA, 23 bp, synthetic construct
  misc_feature 1..23: note = Atg1-R
  source 1..23: mol_type = other DNA
ggaaggttctttggcaccagcac

SEQ ID NO: 15 - DNA, 20 bp, synthetic construct
  misc_feature 1..20: note = Atg8-F
  source 1..20: mol_type = other DNA
ccgcagtaggtggcaaagta

SEQ ID NO: 16 - DNA, 20 bp, synthetic construct
  misc_feature 1..20: note = Atg8-R
  source 1..20: mol_type = other DNA
ggagtcggagaggattgctg

SEQ ID NO: 17 - DNA, 19 bp, synthetic construct
  misc_feature 1..19: note = FOXO-F
  source 1..19: mol_type = other DNA
cggacaaacggctcactct

SEQ ID NO: 18 - DNA, 21 bp, synthetic construct
  misc_feature 1..21: note = FOXO-R
  source 1..21: mol_type = other DNA
ggacccgcatgaatcgactat

SEQ ID NO: 19 - DNA, 21 bp, synthetic construct
  misc_feature 1..21: note = SIRT1-F
  source 1..21: mol_type = other DNA
tgctggcctaatagagtggca

SEQ ID NO: 20 - DNA, 20 bp, synthetic construct
  misc_feature 1..20: note = SIRT1-R
  source 1..20: mol_type = other DNA
ctcagcgccatggaaaatgt

SEQ ID NO: 21 - DNA, 20 bp, synthetic construct
  misc_feature 1..20: note = NADSYN-F
  source 1..20: mol_type = other DNA
gcaaaatgtgcaggctcgaa

SEQ ID NO: 22 - DNA, 20 bp, synthetic construct
  misc_feature 1..20: note = NADSYN-R
  source 1..20: mol_type = other DNA
gcactggagcagtcgtactt

SEQ ID NO: 23 - DNA, 18 bp, synthetic construct
  misc_feature 1..18: note = MRPS5-F
  source 1..18: mol_type = other DNA
gtccggacagtccctcac

SEQ ID NO: 24 - DNA, 21 bp, synthetic construct
  misc_feature 1..21: note = MRPS5-R
  source 1..21: mol_type = other DNA
cccaataaatgacctgccgtc

SEQ ID NO: 25 - DNA, 18 bp, synthetic construct
  misc_feature 1..18: note = SOD3-F
  source 1..18: mol_type = other DNA
agctggaaaggtgcccga

SEQ ID NO: 26 - DNA, 21 bp, synthetic construct
  misc_feature 1..21: note = SOD3-R
  source 1..21: mol_type = other DNA
cttggcgtacatgtctcggat

SEQ ID NO: 27 - protein, 9 aa, Saccharomyces cerevisiae TCI907
MVAKAHSKK